European Patent Application EP 4 628 583 A1, published October 8, 2025. Title: 双环脱碱基核酸类似物以及由它们制备的寡聚化合物. Applicant: 上海舶望制药有限公司. Application CN. The sequence listing filed with the application follows.

SEQUENCE LISTING (35 sequences)

SEQ ID NO: 1 - RNA, 21 nt, synthetic construct
  source 1..21: mol_type = other RNA
aactcaataaagtgctttgaa

SEQ ID NO: 2 - RNA, 21 nt, synthetic construct
  source 1..21: mol_type = other RNA
ttcaaagcactttattgagtt

SEQ ID NO: 3 - RNA, 21 nt, synthetic construct
  source 1..21: mol_type = other RNA
aactcaataaagtgctttgaa

SEQ ID NO: 4 - RNA, 21 nt, synthetic construct
  source 1..21: mol_type = other RNA
ttcaaagcactttattgagtt

SEQ ID NO: 5 - RNA, 22 nt, synthetic construct
  source 1..22: mol_type = other RNA
aactcaataaagtgctttgaat

SEQ ID NO: 6 - RNA, 21 nt, synthetic construct
  source 1..21: mol_type = other RNA
ttcaaagcactttattgagtt

SEQ ID NO: 7 - RNA, 21 nt, synthetic construct
  source 1..21: mol_type = other RNA
aactcaataaagtgctttgaa

SEQ ID NO: 8 - RNA, 21 nt, synthetic construct
  source 1..21: mol_type = other RNA
ttcaaagcactttattgagtt

SEQ ID NO: 9 - RNA, 21 nt, synthetic construct
  source 1..21: mol_type = other RNA
aactcaataaagtgctttgaa

SEQ ID NO: 10 - RNA, 21 nt, synthetic construct
  source 1..21: mol_type = other RNA
ttcaaagcactttattgagtt

SEQ ID NO: 11 - RNA, 21 nt, synthetic construct
  source 1..21: mol_type = other RNA
aactcaataaagtgctttgaa

SEQ ID NO: 12 - RNA, 21 nt, synthetic construct
  source 1..21: mol_type = other RNA
ttcaaagcactttattgagtt

SEQ ID NO: 13 - RNA, 22 nt, synthetic construct
  source 1..22: mol_type = other RNA
aactcaataaagtgctttgaat

SEQ ID NO: 14 - RNA, 21 nt, synthetic construct
  source 1..21: mol_type = other RNA
ttcaaagcactttattgagtt

SEQ ID NO: 15 - RNA, 21 nt, synthetic construct
  source 1..21: mol_type = other RNA
aactcaataaagtgctttgaa

SEQ ID NO: 16 - RNA, 21 nt, synthetic construct
  source 1..21: mol_type = other RNA
ttcaaagcactttattgagtt

SEQ ID NO: 17 - RNA, 21 nt, synthetic construct
  source 1..21: mol_type = other RNA
aactcaataaagtgctttgaa

SEQ ID NO: 18 - RNA, 21 nt, synthetic construct
  source 1..21: mol_type = other RNA
ttcaaagcactttattgagtt

SEQ ID NO: 19 - RNA, 21 nt, synthetic construct
  source 1..21: mol_type = other RNA
aactcaataaagtgctttgaa

SEQ ID NO: 20 - RNA, 21 nt, synthetic construct
  source 1..21: mol_type = other RNA
aactcaataaagtgctttgaa

SEQ ID NO: 21 - RNA, 21 nt, synthetic construct
  source 1..21: mol_type = other RNA
aactcaataaagtgctttgaa

SEQ ID NO: 22 - RNA, 21 nt, synthetic construct
  source 1..21: mol_type = other RNA
aactcaataaagtgctttgaa

SEQ ID NO: 23 - RNA, 21 nt, synthetic construct
  source 1..21: mol_type = other RNA
ttcaaagcactttattgagtt

SEQ ID NO: 24 - RNA, 21 nt, synthetic construct
  source 1..21: mol_type = other RNA
cattttaatcctcactctaaa

SEQ ID NO: 25 - RNA, 21 nt, synthetic construct
  source 1..21: mol_type = other RNA
cattttaatcctcactctaaa

SEQ ID NO: 26 - RNA, 21 nt, synthetic construct
  source 1..21: mol_type = other RNA
cattttaatcctcactctaaa

SEQ ID NO: 27 - RNA, 21 nt, synthetic construct
  source 1..21: mol_type = other RNA
cattttaatcctcactctaaa

SEQ ID NO: 28 - RNA, 21 nt, synthetic construct
  source 1..21: mol_type = other RNA
cattttaatcctcactctaaa

SEQ ID NO: 29 - RNA, 21 nt, synthetic construct
  source 1..21: mol_type = other RNA
cattttaatcctcactctaaa

SEQ ID NO: 30 - RNA, 20 nt, synthetic construct
  source 1..20: mol_type = other RNA
ttagagtgaggattaaaatg

SEQ ID NO: 31 - RNA, 22 nt, synthetic construct
  source 1..22: mol_type = other RNA
ttagagtgaggattaaaatgag

SEQ ID NO: 32 - RNA, 20 nt, synthetic construct
  source 1..20: mol_type = other RNA
ttagagtgaggattaaaatg

SEQ ID NO: 33 - RNA, 20 nt, synthetic construct
  source 1..20: mol_type = other RNA
ttagagtgaggattaaaatg

SEQ ID NO: 34 - RNA, 22 nt, synthetic construct
  source 1..22: mol_type = other RNA
ttagagtgaggattaaaatgag

SEQ ID NO: 35 - RNA, 22 nt, synthetic construct
  source 1..22: mol_type = other RNA
ttagagtgaggattaaaatgag